European Patent Specification EP 3 897 683 B1, published November 15, 2023. Title: Cosmetic, pharmaceutical and nutraceutical use of an extract derived from Cannabis sativa cell cultures. Applicant: Arterra Bioscience Srl. The sequence listing filed with the application follows.

SEQUENCE LISTING (12 sequences)

SEQ ID NO: 1 - DNA, 20 bp, Unknown
  None
gcaggtgtggtgttcatccc

SEQ ID NO: 2 - DNA, 20 bp, Unknown
  None
gggcattctcaccaagttct

SEQ ID NO: 3 - DNA, 20 bp, Unknown
  None
gccaccggagcactccataa

SEQ ID NO: 4 - DNA, 24 bp, Unknown
  None
ctcttcaaaaacttctccacaacc

SEQ ID NO: 5 - DNA, 22 bp, Unknown
  None
atgagcactgaaagcatgatcc

SEQ ID NO: 6 - DNA, 21 bp, Unknown
  None
tcataccagggcttggcctca

SEQ ID NO: 7 - DNA, 23 bp, Unknown
  None
actgcagccccagctgcatccta

SEQ ID NO: 8 - DNA, 20 bp, Unknown
  None
aggtgatgacacttgtccag

SEQ ID NO: 9 - DNA, 20 bp, Unknown
  None
gaagctcatcctgttcatcg

SEQ ID NO: 10 - DNA, 20 bp, Unknown
  None
atcagcaggaaggcatagct

SEQ ID NO: 11 - DNA, 20 bp, Unknown
  None
ggcaagcgctcctactccat

SEQ ID NO: 12 - DNA, 20 bp, Unknown
  None
tcactcgcccttcttgtagg